European Patent Application EP 4 563 588 A1, published June 4, 2025. Title: Composition of Antibacterial Protein for Treating Bovine Mastitis. Applicant: iNtRON Biotechnology, Inc. The sequence listing filed with the application follows.

SEQUENCE LISTING (2 sequences)

SEQ ID NO: 1 - protein, 325 aa, Artificial Sequence
MAKTQAEINKRLDAYAKGTVDSPYRIKKATSYDPSFGVMEAGAIDADGYYHAQCQDLITDYVLWLTDNKVRTWGNAKDQIKQSYGTGFKIHENKPSTVPKKGWIAVFTSGSYQQWGHIGIVYDGGNTSTFTILEQNWNGYANKKPTKRVDNYYGLTHFIEIPVKAGTTVKKETAKKSASKTPAPKKKATLKVSKNHINYTMDKRGKKPEGMVIHNDAGRSTPATRPVTGSWKKNQYGTWYKPENATFVNGNQPIVTRIGSPFLNAPVGGNLPAGATIVYDEVSIQAGHIWIGYNAYNGNRVYSPVRTCQGVPPNHIPGVAWGVFK

SEQ ID NO: 2 - DNA, 5045 bp, Artificial Sequence
  source 1..5045: mol_type = other DNA
aagaaaccaattgtccatattgcatcagacattgccgtcactgcgtcttttactggctcttctcgctaaccaaaccggtaaccccgcttattaaaagcattctgtaacaaagcgggaccaaagccatgacaaaaacgcgtaacaaaagtgtctataatcacggcagaaaagtccacattgattatttgcacggcgtcacactttgctatgccatagcatttttatccataagattagcggatcctacctgacgctttttatcgcaactctctactgtttctccatacccgtttttttgggctagaaataattttgtttaactttaagaaggagatatacatccatggctaagactcaagcagaaataaataaacgtttagacgcttatgcaaaaggtacagtagacagtccttatagaattaaaaaagctacaagctatgacccatcgtttggtgtaatggaagcaggagcaattgacgcagatggttactatcatgcacagtgccaagacttaattactgattatgtattatggttaacagataataaagttagaacttggggtaatgctaaagaccaaatcaaacaaagttatggtactggatttaaaatacatgaaaataaaccttctacagtacctaaaaaaggatggattgctgtatttacatccggtagttatcagcaatggggtcacataggtattgtatatgatggaggtaatacttctacatttactattttagagcaaaactggaacggttacgctaataaaaaacctacaaaacgtgtagataattattacggattaactcattttattgagatacctgtaaaagcaggaactactgttaaaaaagaaacagctaagaaaagtgcaagtaaaacacctgcacctaaaaagaaagcaacactaaaagtttctaagaaccatattaactatacaatggataaacgtggtaagaaacctgaaggaatggtaatacacaacgatgcaggtcgttctacaccggcaactagaccagtaacaggctcttggaaaaagaaccagtacggaacttggtacaaaccggaaaatgcaacatttgttaatggtaaccaacctatagtaactagaataggttctccattcttaaatgctccagtaggaggtaacttaccggcaggagctacaattgtatatgacgaagttagtatccaagcaggtcacatttggataggttacaatgcttacaatggtaacagagtatatagccctgttagaacttgtcaaggagttccacctaatcatatacctggggttgcctggggagtattcaaataagcggccgcaagggcgagcttgaaggtaagcctatccctaaccctctcctcggtctcgattctacgcgtaccggtcatcatcaccatcaccattgagtttaaacggtctccagcttggctgttttggcggatgagagaagattttcagcctgatacagattaaatcagaacgcagaagcggtctgataaaacagaatttgcctggcggcagtagcgcggtggtcccacctgaccccatgccgaactcagaagtgaaacgccgtagcgccgatggtagtgtggggtctccccatgcgagagtagggaactgccaggcatcaaataaaacgaaaggctcagtcgaaagactgggcctttcgttttatctgttgtttgtcggtgaacgctctcctgagtaggacaaatccgccgggagcggatttgaacgttgcgaagcaacggcccggagggtggcgggcaggacgcccgccataaactgccaggcatcaaattaagcagaaggccatcctgacggatggcctttttgcgtttctacaaactcttttgtttatttttctaaatacattcaaatatgtatccgctcatgagattatcaaaaaggatcttcacctagatccttttaaattaaaaatgaagttttaaatcaatctaaagtatatatgagtaaacttggtctgacagttaggcgtcgcttggtcggtcatttcgaaccccagagtcccgctcagaagaactcgtcaagaaggcgatagaaggcgatgcgctgcgaatcgggagcggcgataccgtaaagcacgaggaagcggtcagcccattcgccgccaagctcttcagcaatatcacgggtagccaacgctatgtcctgatagcggtccgccacacccagccggccacagtcgatgaatccagaaaagcggccattttccaccatgatattcggcaagcaggcatcgccatgtgtcacgacgagatcctcgccgtcgggcatgcgcgccttgagcctggcgaacagttcggctggcgcgagcccctgatgctcttcgtccagatcatcctgatcgacaagaccggcttccatccgagtacgtgctcgctcgatgcgatgtttcgcttggtggtcgaatgggcaggtagccggatcaagcgtatgcagccgccgcattgcatcagccatgatggatactttctcggcaggagcaaggtgagatgacaggagatcctgccccggcacttcgcccaatagcagccagtcccttcccgcttcagtgacaacgtcgagcacagctgcgcaaggaacgcccgtcgtggccagccacgatagccgcgctgcctcgtcctgcagttcattcagggcaccggacaggtcggtcttgacaaaaagaaccgggcgcccctgcgctgacagccggaacacggcggcatcagagcagccgattgtcagttgtgcccagtcatagccgaatagcctctccacccaagcggccggagaacctgcgtgcaatccatcttgttcaatcatactcttcctttttcaatattattgaagcatttatcagggttattgtctcatgaccaaaatcccttaacgtgagttttcgttccactgagcgtcagaccccgtagaaaagatcaaaggatcttcttgagatcctttttttctgcgcgtaatctgctgcttgcaaacaaaaaaaccaccgctaccagcggtggtttgtttgccggatcaagagctaccaactctttttccgaaggtaactggcttcagcagagcgcagataccaaatactgtccttctagtgtagccgtagttaggccaccacttcaagaactctgtagcaccgcctacatacctcgctctgctaatcctgttaccagtggctgctgccagtggcgataagtcgtgtcttaccgggttggactcaagacgatagttaccggataaggcgcagcggtcgggctgaacggggggttcgtgcacacagcccagcttggagcgaacgacctacaccgaactgagatacctacagcgtgagctatgagaaagcgccacgcttcccgaagggagaaaggcggacaggtatccggtaagcggcagggtcggaacaggagagcgcacgagggagcttccagggggaaacgcctggtatctttatagtcctgtcgggtttcgccacctctgacttgagcgtcgatttttgtgatgctcgtcaggggggcggagcctatggaaaaacgccagcaacgcggcctttttacggttcctggcattttgctggccttttgctcacatgttctttcctgcgttatcccctgattctgtggataaccgtattaccgcctttgagtgagctgataccgctcgccgcagccgaacgaccgagcgcagcgagtcagtgagcgaggaagcggaagagcgcctgatgcggtattttctccttacgcatctgtgcggtatttcacaccgcatatggtgcactctcagtacaatctgctctgatgccgcatagttaagccagtatacactccgctatcgctacgtgactgggtcatggctgcgccccgacacccgccaacacccgctgacgcgccctgacgggcttgtctgctcccggcatccgcttacagacaagctgtgaccgtctccgggagctgcatgtgtcagaggttttcaccgtcatcaccgaaacgcgcgaggcagcagatcaattcgcgcgcgaaggcgaagcggcatgcataatgtgcctgtcaaatggacgaagcagggattctgcaaaccctatgctactccgtcaagccgtcaattgtctgattcgttaccaattatgacaacttgacggctacatcattcactttttcttcacaaccggcacggaactcgctcgggctggccccggtgcattttttaaatacccgcgagaaatagagttgatcgtcaaaaccaacattgcgaccgacggtggcgataggcatccgggtggtgctcaaaagcagcttcgcctggctgatacgttggtcctcgcgccagcttaagacgctaatccctaactgctggcggaaaagatgtgacagacgcgacggcgacaagcaaacatgctgtgcgacgctggcgatatcaaaattgctgtctgccaggtgatcgctgatgtactgacaagcctcgcgtacccgattatccatcggtggatggagcgactcgttaatcgcttccatgcgccgcagtaacaattgctcaagcagatttatcgccagcagctccgaatagcgcccttccccttgcccggcgttaatgatttgcccaaacaggtcgctgaaatgcggctggtgcgcttcatccgggcgaaagaaccccgtattggcaaatattgacggccagttaagccattcatgccagtaggcgcgcggacgaaagtaaacccactggtgataccattcgcgagcctccggatgacgaccgtagtgatgaatctctcctggcgggaacagcaaaatatcacccggtcggcaaacaaattctcgtccctgatttttcaccaccccctgaccgcgaatggtgagattgagaatataacctttcattcccagcggtcggtcgataaaaaaatcgagataaccgttggcctcaatcggcgttaaacccgccaccagatgggcattaaacgagtatcccggcagcaggggatcattttgcgcttcagccatacttttcatactcccgccattcagag